European Patent Application EP 4 810 624 A1, published September 23, 2026. Title: LINEAR DNA PRODUCTS AND METHODS FOR THE PRODUCTION THEREOF. Applicant: 4basebio UK Ltd. The sequence listing filed with the application follows.

SEQUENCE LISTING (12 sequences)

SEQ ID NO: 1 - DNA, 41 bp, synthetic construct
  source 1..41: mol_type = other DNA
agggctaacatttgttggccactcaggccaacaaatgttag

SEQ ID NO: 2 - DNA, 20 bp, synthetic construct
  source 1..20: mol_type = other DNA
  modified_base 16..20: mod_base = OTHER; note = phosphorothioated nucleotide
aaaaaaaaaaaaaaaaaaaa

SEQ ID NO: 3 - DNA, 16 bp, synthetic construct
  source 1..16: mol_type = other DNA
  modified_base 2..6: mod_base = OTHER; note = phosphorothioated nucleotide
tttttttttttttttt

SEQ ID NO: 4 - DNA, 33 bp, synthetic construct
  source 1..33: mol_type = other DNA
  modified_base 29..33: mod_base = OTHER; note = phosphorothioated nucleotide
agcgatggtctcaaaaaaaaaaaaaaaaaaaaa

SEQ ID NO: 5 - DNA, 33 bp, synthetic construct
  source 1..33: mol_type = other DNA
  modified_base 2..6: mod_base = OTHER; note = phosphorothioated nucleotide
tttttttttttttttttttttgagaccatcgct

SEQ ID NO: 6 - DNA, 20 bp, synthetic construct
  source 1..20: mol_type = other DNA
  modified_base 2..6: mod_base = OTHER; note = phosphorothioated nucleotides
tttttttttttttttttttt

SEQ ID NO: 7 - DNA, 34 bp, synthetic construct
  source 1..34: mol_type = other DNA
  modified_base 30..34: mod_base = OTHER; note = phosphorothioated nucleotide
ggcattgcgtctcaaaaaaaaaaaaaaaaaaaaa

SEQ ID NO: 8 - DNA, 38 bp, synthetic construct
  source 1..38: mol_type = other DNA
  modified_base 2..6: mod_base = OTHER; note = phosphorothioated nucleotide
tttttttttttttttttttttttttgagacgcaatgcc

SEQ ID NO: 9 - DNA, 34 bp, synthetic construct
  source 1..34: mol_type = other DNA
  modified_base 33: mod_base = OTHER; note = locked nucleic acid
ggcattgggtctcaaaaaaaaaaaaaaaaaaaaa

SEQ ID NO: 10 - DNA, 34 bp, synthetic construct
  source 1..34: mol_type = other DNA
  modified_base 2..6: mod_base = OTHER; note = phosphorothioated nucleotide
tttttttttttttttttttttgagacccaatgcc

SEQ ID NO: 11 - DNA, 20 bp, synthetic construct
  source 1..20: mol_type = other DNA
ctgtttaaatcactgaggta

SEQ ID NO: 12 - DNA, 20 bp, synthetic construct
  source 1..20: mol_type = other DNA
ctctttcgtttgggttgttt